European Patent Application EP 4 410 975 A1, published August 7, 2024. Title: METHOD FOR PRODUCING CELL HAVING DNA DELETION SPECIFIC TO ONE OF HOMOLOGOUS CHROMOSOMES. Applicant: OSAKA UNIVERSITY. The sequence listing filed with the application follows.

SEQUENCE LISTING (21 sequences)

SEQ ID NO: 1 - DNA, 23 bp, synthetic construct
  source 1..23: mol_type = other DNA
cgtctcggagcaggcaggcgggg

SEQ ID NO: 2 - DNA, 23 bp, synthetic construct
  source 1..23: mol_type = other DNA
agcttcccatctatacctcctgg

SEQ ID NO: 3 - DNA, 23 bp, synthetic construct
  source 1..23: mol_type = other DNA
gaggtaggttgatcttgtgtggg

SEQ ID NO: 4 - DNA, 23 bp, synthetic construct
  source 1..23: mol_type = other DNA
tcccaccgaaggccacacgccgg

SEQ ID NO: 5 - DNA, 23 bp, synthetic construct
  source 1..23: mol_type = other DNA
ctcgcagaactccagggaactgg

SEQ ID NO: 6 - DNA, 23 bp, synthetic construct
  source 1..23: mol_type = other DNA
cccctggctttcctggcactggg

SEQ ID NO: 7 - DNA, 23 bp, synthetic construct
  source 1..23: mol_type = other DNA
tggcagccacggcttccccctgg

SEQ ID NO: 8 - DNA, 22 bp, synthetic construct
  source 1..22: mol_type = other DNA
gcctttcccataggtgctaact

SEQ ID NO: 9 - DNA, 28 bp, synthetic construct
  source 1..28: mol_type = other DNA
aacaaaacacactctggaagatggaacc

SEQ ID NO: 10 - DNA, 25 bp, synthetic construct
  source 1..25: mol_type = other DNA
cacaaggcacaggacacactgttag

SEQ ID NO: 11 - DNA, 28 bp, synthetic construct
  source 1..28: mol_type = other DNA
aacaaaacacactctggaagatggaacc

SEQ ID NO: 12 - DNA, 22 bp, synthetic construct
  source 1..22: mol_type = other DNA
gagtactcgggttcgtgaactt

SEQ ID NO: 13 - DNA, 22 bp, synthetic construct
  source 1..22: mol_type = other DNA
gcagcttcccatctatacctcc

SEQ ID NO: 14 - DNA, 22 bp, synthetic construct
  source 1..22: mol_type = other DNA
aagccctcacgtctcaataacc

SEQ ID NO: 15 - DNA, 22 bp, synthetic construct
  source 1..22: mol_type = other DNA
gctttaagcagaccagtgggta

SEQ ID NO: 16 - DNA, 21 bp, synthetic construct
  source 1..21: mol_type = other DNA
ttttctggacgagggcctttc

SEQ ID NO: 17 - DNA, 22 bp, synthetic construct
  source 1..22: mol_type = other DNA
cttccaagtcagcgagggaaaa

SEQ ID NO: 18 - DNA, 21 bp, synthetic construct
  source 1..21: mol_type = other DNA
cctcatggttccttttgcttg

SEQ ID NO: 19 - DNA, 20 bp, synthetic construct
  source 1..20: mol_type = other DNA
ggtgggaaaatcgcttgaat

SEQ ID NO: 20 - DNA, 18 bp, synthetic construct
  source 1..18: mol_type = other DNA
tgaacactgagcctgctt

SEQ ID NO: 21 - DNA, 17 bp, synthetic construct
  source 1..17: mol_type = other DNA
cgtttattttcttgttg